European Patent Specification EP 4 090 327 B1, published March 5, 2025. Title: USE OF FXR AGONIST FOR TREATING AN INFECTION BY HEPATITIS D VIRUS. Applicant: INSERM et al. The sequence listing filed with the application follows.

SEQUENCE LISTING (6 sequences)

SEQ ID NO: 1 - DNA, 20 bp, artificial
  primer HDV-F
gcctctccttgtcggtgaat

SEQ ID NO: 2 - DNA, 20 bp, artificial
  primer HDV-R
cctggctggggaacatcaaa

SEQ ID NO: 3 - DNA, 23 bp, artificial
  primer HBV-F
agctactgtggagttactctcgt

SEQ ID NO: 4 - DNA, 22 bp, artificial
  primer HBV-R
caaagaattgcttgcctgagtg

SEQ ID NO: 5 - DNA, 20 bp, artificial
  primer S9-F
ccgcgtgaagaggaagaatg

SEQ ID NO: 6 - DNA, 21 bp, artificial
  primer S9-R
ttggcaggaaaacgagacaat